European Patent Specification EP 3 721 227 B1, published February 8, 2023. Title: Olfactory receptor involved in the perception of musk fragrance and the use thereof. Applicant: ChemCom S.A. The sequence listing filed with the application follows.

SEQUENCE LISTING (12 sequences)

SEQ ID NO: 1 - DNA, 975 bp, Homo sapiens
atggctgtaggaaggaacaacacaattgtgacaaaattcattctcctgggactttcagaccatcctcaaatgaagattttccttttcatgttatttctggggctctacctcctgacgttggcctggaacttaagcctcattgccctcattaagatggactctcacctgcacatgcccatgtacttcttcctcagtaacctgtccttcctggacatctgctatgtgtcctccaccgcccctaagatgctgtctgacatcatcacagagcagaaaaccatttcctttgttggctgtgccactcagtactttgtcttctgtgggatggggctgactgaatgctttctcctggcagctatggcctatgaccggtatgctgcaatctgcaaccccttgctttacacagtcctcatatcccatacactttgtttaaagatggtggttggcgcctatgtgggtggattccttagttctttcattgaaacatactctgtctatcagcatgatttctgtgggccctatatgatcaaccactttttctgtgacctccctccagtcctggctctgtcctgctctgataccttcaccagcgaggtggtgaccttcatagtcagtgttgtcgttggaatagtgtctgtgctagtggtcctcatctcttatggttacattgttgctgctgttgtgaagatcagctcagctacaggtaggacaaaggccttcagcacttgtgcctctcacctgactgctgtgaccctcttctatggttctggattcttcatgtacatgcgacccagttccagctactccctaaacagggacaaggtggtgtccatattctatgccttggtgatccccgtggtgaatcccatcatctacagttttaggaataaggagattaaaaatgccatgaggaaagccatggaaagggaccccgggatttctcacggtggaccattcatttttatgaccttgggctaa

SEQ ID NO: 2 - protein, 324 aa, Homo sapiens
MAVGRNNTIVTKFILLGLSDHPQMKIFLFMLFLGLYLLTLAWNLSLIALIKMDSHLHMPMYFFLSNLSFLDICYVSSTAPKMLSDIITEQKTISFVGCATQYFVFCGMGLTECFLLAAMAYDRYAAICNPLLYTVLISHTLCLKMVVGAYVGGFLSSFIETYSVYQHDFCGPYMINHFFCDLPPVLALSCSDTFTSEVVTFIVSVVVGIVSVLVVLISYGYIVAAVVKISSATGRTKAFSTCASHLTAVTLFYGSGFFMYMRPSSSYSLNRDKVVSIFYALVIPVVNPIIYSFRNKEIKNAMRKAMERDPGISHGGPFIFMTLG

SEQ ID NO: 3 - DNA, 975 bp, Homo sapiens
atggctgtaggaaggaacaacacaattgtgacaaaattcattctcctgggactttcagaccatcctcaaatgaagattttccttttcatgttatttctggggctctacctcctgacgttggcctggaacttaagcctcattgccctcattaagatggactctcacctgcacatgcccatgtacttcttcctcagtaacctgtccttcctggacatctgctatgtgtcctccaccgcccctaagatgctgtctgacatcatcacagagcagaaaaccatttcctttgttggctgtgccactcagtactttgtcttctgtgggatggggctgactgaatgctttctcctggcagctatggcctatgaccggtatgctgcaatctgcaaccccttgctttacacagtcctcatatcccatacactttgtttaaagatggtggttggcgcctatgtgggtggattccttagttctttcattgaaacatactctgtctatcagcatgatttctgtgggctctatatgatcaaccactttttctgtgacctccctccagtcctggctctgtcctgctctgataccttcaccagcgaggtggtgaccttcatagtcagtgttgtcgttggaatagtgtctgtgctagtggtcctcatctcttatggttacattgttgctgctgttgtgaagatcagctcagctacaggtaggacaaaggccttcagcacttgtgcctctcacctgactgctgtgaccctcttctatggttctggattcttcatgtacatgcgacccagttccagctactccctaaacagggacaaggtggtgtccatattctatgccttggtgatccccgtggtgaatcccatcatctacagttttaggaataaggagattaaaaatgccatgaggaaagccatggaaagggaccccgggatttctcacggtggaccattcatttttatgaccttgggctaa

SEQ ID NO: 4 - protein, 324 aa, Homo sapiens [sequence omitted]

SEQ ID NO: 5 - protein, 7 aa, artificial sequence
  MARCKS peptide
  MOD_RES (1)..(1): ACETYLATION
  MOD_RES (6)..(6): AMIDATION
FKKSFKL

SEQ ID NO: 6 - protein, 13 aa, Artificial seqence
  Src-related peptide
RRLIEDAEYAARG

SEQ ID NO: 7 - protein, 311 aa, Homo sapiens
MTGGGNITEITYFILLGFSDFPRIIKVLFTIFLVIYITSLAWNLSLIVLIRMDSHLHTPMYFFLSNLSFIDVCYISSTVPKMLSNLLQGQQTITFVGCIIQYFIFSTMGLSESCLMTAMAYDRYAAICNPLLYSSIMSPTLCVWMVLGAYMTGLTASLFQIGALLQLHFCGSNVIRHFFCDMPQLLILSCTDTFFVQVMTAILTMFFGIASALVIMISYGYIGISIMKITSAKGRSKAFNTCASHLTAVSLFYTSGIFVYLSSSSGGSSSFDRFASVFYTVVIPMLNPLIYSLRNKEIKDALKRLQKRKCC

SEQ ID NO: 8 - protein, 315 aa, Homo sapiens
MEIVSTGNETITEFVLLGFYDIPELHFLFFIVFTAVYVFIIIGNMLIIVAVVSSQRLHKPMYIFLANLSFLDILYTSAVMPKMLEGFLQEATISVAGCLLQFFIFGSLATAECLLLAVMAYDRYLAICYPLHYPLLMGPRRYMGLVVTTWLSGFVVDGLVVALVAQLRFCGPNHIDQFYCDFMLFVGLACSDPRVAQVTTLILSVFCLTIPFGLILTSYARIVVAVLRVPAGASRRRAFSTCSSHLAVVTTFYGTLMIFYVAPSAVHSQLLSKVFSLLYTVVTPLFNPVIYTMRNKEVHQALRKILCIKQTETLD

SEQ ID NO: 9 - protein, 315 aa, Homo sapiens
MSITKAWNSSSVTMFILLGFTDHPELQALLFVTFLGIYLTTLAWNLALIFLIRGDTHLHTPMYFFLSNLSFIDICYSSAVAPNMLTDFFWEQKTISFVGCAAQFFFFVGMGLSECLLLTAMAYDRYAAISSPLLYPTIMTQGLCTRMVVGAYVGGFLSSLIQASSIFRLHFCGPNIINHFFCDLPPVLALSCSDTFLSQVVNFLVVVTVGGTSFLQLLISYGYIVSAVLKIPSAEGRWKACNTCASHLMVVTLLFGTALFVYLRPSSSYLLGRDKVVSVFYSLVIPMLNPLIYSLRNKEIKDALWKVLERKKVFS

SEQ ID NO: 10 - protein, 310 aa, Artificial sequence
  chimeric receptor OR5A2_variant 1
MTKNQTWVTEFILLGFPLSLRIQMLLSGLFSLLYVFTLLGNGAILGLIWLDSRLHTPMYFFLSNLSFLDICYVSSTAPKMLSDIITEQKTISFVGCATQYFVFCGMGLTECFLLAAMAYDRYAAICNPLLYTVLISHTLCLKMVVGAYVGGFLSSFIETYSVYQHDFCGPYMINHFFCDLPPVLALSCSDTFTSEVVTFIVSVVVGIVSVLVVLISYGYIVAAVVKISSATGRTKAFSTCASHLTAVTLFYGSGFFMYMRPSSSYSLNRDKVVSIFYALVIPVVNPLIYSLRNAEVKGALKRVLWKQRSK

SEQ ID NO: 11 - protein, 228 aa, Homo sapiens
PMYFFLSNLSFLDICYVSSTAPKMLSDIITEQKTISFVGCATQYFVFCGMGLTECFLLAAMAYDRYAAICNPLLYTVLISHTLCLKMVVGAYVGGFLSSFIETYSVYQHDFCGPYMINHFFCDLPPVLALSCSDTFTSEVVTFIVSVVVGIVSVLVVLISYGYIVAAVVKISSATGRTKAFSTCASHLTAVTLFYGSGFFMYMRPSSSYSLNRDKVVSIFYALVIPVV

SEQ ID NO: 12 - protein, 311 aa, Homo sapiens [sequence omitted]